European Patent Application EP 4 170 020 A1, published April 26, 2023. Title: Immunocompetent cells expressing chimeric antigen-receptor. Applicant: Kyoto University. The sequence listing filed with the application follows.

SEQUENCE LISTING (15 sequences)

SEQ ID NO: 1 - protein, 400 aa, Homo sapiens
  SIGNAL (1)..(23): human IL-2 lead sequence
  PEPTIDE (24)..(137): human IL-15
  PEPTIDE (138)..(161): Peptide Linker
  PEPTIDE (162)..(400): human IL-15Ra
MYRMQLLSCIALSLALVTNSATSNWVNVISDLKKIEDLIQSMHIDATLYTESDVHPSCKVTAMKCFLLELQVISLESGDASIHDTVENLIILANNSLSSNGNVTESGCKECEELEEKNIKEFLQSFVHIVQMFINTSSGGGSGGGGSGGGGSGGGGSGGGSLQITCPPPMSVEHADIWVKSYSLYSRERYICNSGFKRKAGTSSLTECVLNKATNVAHWTTPSLKCIRDPALVHQRPAPPSTVTTAGVTPQPESLSPSGKEPAASSPSSNNTAATTAAIVPGSQLMPSKSPSTGTTEISSHESSHGTPSQTTAKNWELTASASHQPPGVYPQGHSDTTVAISTSTVLLCGLSAVSLLACYLKSRQTPPLASVEMEAMEALPVTWGTSSRDEDLENCSHHL

SEQ ID NO: 2 - DNA, 39 bp, Artificial Sequence
  gRNA sequence for DGKa
gatgatgcgagtggctgaatacctggattgggatgtgtc

SEQ ID NO: 3 - DNA, 36 bp, Artificial Sequence
  gRNA sequence for DGKz
ctggggccccgtgcagcgagtcagagcggcagatcc

SEQ ID NO: 4 - DNA, 57 bp, Artificial Sequence
  DGKa gRNA target-fwd
gagaccacttggatccgagtggctgaatacctggatgttttagagctagaaatagca

SEQ ID NO: 5 - DNA, 93 bp, Artificial Sequence
  gRNA-Universal-rev
gcccgggtttgaattcaaaaaaagcaccgactcggtgccactttttcaagttgataacggactagccttattttaacttgctatttctagctc

SEQ ID NO: 6 - DNA, 57 bp, Artificial Sequence
  DGKz gRNA target-fwd
gagaccacttggatccggccgctctgactcgctgcagttttagagctagaaatagca

SEQ ID NO: 7 - DNA, 67 bp, Artificial Sequence
  T7-DGKa-IVT-fwd
gaaattaatacgactcactataggctctcaagctgagtgggtccgttttagagctagaaatagcaag

SEQ ID NO: 8 - DNA, 79 bp, Artificial Sequence
  sgRNA+85 rev primer
aaagcaccgactcggtgccactttttcaagttgataacggactagccttattttaacttgctatttctagctctaaaac

SEQ ID NO: 9 - DNA, 67 bp, Artificial Sequence
  T7-DGKz-IVT-fwd
gaaattaatacgactcactataggacgagcactcaccagcatccgttttagagctagaaatagcaag

SEQ ID NO: 10 - DNA, 51 bp, Homo sapiens
agatgatgcgagtggctgaatacctggattgggatgtgtctgagctgaggc

SEQ ID NO: 11 - DNA, 35 bp, Homo sapiens
agatgatgcgagtggctgaatacctgagctgaggc

SEQ ID NO: 12 - DNA, 50 bp, Homo sapiens
agatgatgcgagtggctgaatacctgattgggatgtgtctgagctgaggc

SEQ ID NO: 13 - DNA, 61 bp, Homo sapiens
gtcgggcctccagcacctggccccccctccgcccacccctggggccccgtgcagcgagtca

SEQ ID NO: 14 - DNA, 27 bp, Homo sapiens
gtcgggcctccagcacctggcgagtca

SEQ ID NO: 15 - DNA, 62 bp, Homo sapiens
gtcgggcctccagcacctggccccccctccgcccacccctggggccccgtgcaagcgagtca